European Patent Application EP 4 640 226 A1, published October 29, 2025. Title: 克里斯滕森菌或包含其的组合物在预防或治疗肿瘤中的用途以及包含其的药物. Applicant: 慕恩（广州）生物科技有限公司. The sequence listing filed with the application follows.

SEQUENCE LISTING (3 sequences)

SEQ ID NO: 1 - RNA, 1376 nt, Christensenella sp.
  source 1..1376: mol_type = other RNA
tcgaacgaagttgctctttgtgaagccctcgggtggaactgcgagtatacttagtggcggacgggtgagtaacgcgtgagcaatctgccctgcaatgggggacaacagttggaaacgactgctaataccgcatgagaccacgaaaccgcatggttttgaggtaaaaggatttattcgatgcaggatgagctcgcgtcccattagatagttggtgaggtaacggcccaccaagtcaacgatgggtagccgacctgagagggtgatcggccacactggaactgagacacggtccagactcctacgggaggcagcagtggggaatattgggcaatgggggaaaccctgacccagcaacgccgcgtgagggaagaaggtcttcggattgtaaacctttgtcctatgggacgaaacaaatgacggtaccataggaggaagctccggctaactacgtgccagcagccgcggtaatacgtagggagcaagcgttgtccggaattactgggcgtaaagggtgcgtaggtggctatgtaagtcagatgtgaaagaccggggcttaaccccggggttgcatttgaaactgtgtggcttgagtacaggagagggaagtggaattcctagtgtagcggtgaaatgcgtagatattaggaggaacaccagtggcgaaggcgactttctggactgtaactgacactgaagcacgaaagcgtggggagcaaacaggattagataccctggtagtccacgccgtaaacgatggatactaggtgtggggcccgatagggttccgtgccgaagctaacgcattaagtatcccgcctggggagtacgatcgcaaggttgaaactcaaaggaattgacgggggcccgcacaagcagcggagcatgtggtttaattcgaagcaacgcgaagaaccttaccaaggcttgacatcctctgacgactgtagagatacagtttcccttcggggcagagagacaggtggtgcatggttgtcgtcagctcgtgtcgtgagatgttgggttaagtcccgcaacgagcgcaacccttattgctagttgccagcgcgtaaaggcgggaactctagtgagactgccggggacaactcggaggaaggtggggacgacgtcaaatcatcatgccccttatgtcttgggctacacacgtgctacaatggccggtacaaagggcagcgaacccgtaaggggaagcgaatctcaaaaagccggtcccagttcggattgtgggctgcaacccgcccacatgaagtcggagttgctagtaatcgcgaatcagcatgtcgcggtgaatgcgttcccgggccttgtacacaccgcccgtcacaccacggaagttgggagcacccgaagccagtagg

SEQ ID NO: 2 - DNA, 20 bp, synthetic construct
  source 1..20: mol_type = other DNA
agagtttgatcatggctcag

SEQ ID NO: 3 - DNA, 22 bp, synthetic construct
  source 1..22: mol_type = other DNA
tagggttaccttgttacgactt